European Patent Application EP 4 663 660 A1, published December 17, 2025. Title: TRISPECIFIC ANTIGEN-BINDING MOLECULE AND USE THEREOF. Applicant: Shanghai Qilu Pharmaceutical Research and Development Centre Ltd. The sequence listing filed with the application follows.

SEQUENCE LISTING (42 sequences)

SEQ ID NO: 1 - protein, 345 aa, Homo sapiens
MYKDCIESTGDYFLLCDAEGPWGIILESLAILGIVVTILLLLAFLFLMRKIQDCSQWNVLPTQLLFLLSVLGLFGLAFAFIIELNQQTAPVRYFLFGVLFALCFSCLLAHASNLVKLVRGCVSFSWTTILCIAIGCSLLQIIIATEYVTLIMTRGMMFVNMTPCQLNVDFVVLLVYVLFLMALTFFVSKATFCGPCENWKQHGRLIFITVLFSIIIWVVWISMLLRGNPQFQRQPQWDDPVVCIALVTNAWVFLLLYIVPELCILYRSCRQECPLQGNACPVTAYQHSFQVENQELSRARDSDGAEEDVALTSYGTPIQPQTVDPTQECFIPQAKLSPQQDAGGV

SEQ ID NO: 2 - protein, 344 aa, Macaca fascicularis
MYKDCIESTGDYFLPCDSEGPWGIVLESLAILGIVVTILLLLAFLFLMRKIQDCSQWNVLPTQLLFLLSVLGLFGLAFAFIIQLNQQTAPVRYFLFGVLFALCFSCLLAHASNLVKLVRGRVSFSWTTILCIAIGCSLLQVIIAIEYVTLIMTRGMMFVHMTPYQLNVDFVVLLVYVLFLMALTFFVSKATFCGPCENWKQHGRLIFITVLFSIIIWVVWISMLLRGNPQFQRQPQWDDPVVCIALVTNAWVFLLLYIVPELCILYRSCRQECPSQGHACPVTAYQRSFQVENQELSRARDSDGAEEDVALTSFGTPIQPQTVDPTQECFIPRAKLSPQQDAGV

SEQ ID NO: 3 - protein, 184 aa, Homo sapiens
MLQMAGQCSQNEYFDSLLHACIPCQLRCSSNTPPLTCQRYCNASVTNSVKGTNAILWTCLGLSLIISLAVFVLMFLLRKINSEPLKDEFKNTGSGLLGMANIDLEKSRTGDEIILPRGLEYTVEECTCEDCIKSKPKVDSDHCFPLPAMEEGATILVTTKTNDYCKSLPAALSATEIEKSISAR

SEQ ID NO: 4 - protein, 183 aa, Macaca fascicularis
MLQMARQCSQNEYFDSLLHDCKPCQLRCSSTPPLTCQRYCNASMTNSVKGMNAILWTCLGLSLIISLAVFVLTFLLRKMSSEPLKDEFKNTGSGLLGMANIDLEKGRTGDEIVLPRGLEYTVEECTCEDCIKNKPKVDSDHCFPLPAMEEGATILVTTKTNDYCNSLSAALSVTEIEKSISAR

SEQ ID NO: 5 - protein, 708 aa, synthetic construct
QVQLVQSGAEVKKPGASVKVSCKASGFTFRSSYISWVRQAPGQGLEWIAWIYAGSGNADYNQKFTGRVTMTVDTSTSTVYMELSSLRSEDTAVYYCARHYDPPHYFDYWGQGTLVTVSSASTKGPSVFPLAPSSKSTSGGTAALGCLVKDYFPEPVTVSWNSGALTSGVHTFPAVLQSSGLYSLSSVVTVPSSSLGTQTYICNVNHKPSNTKVDKKVEPKSCGGGGSEVKLVESGGGLVQPGGSLKLSCAASGFTFNTYAMNWVRQAPGKGLEWVARIRSKYNNYATYYADSVKDRFTISRDDAKNTLYLQMNNLRTEDTAVYYCVRHGNFGNSYVSWFAYWGQGTLVTVSSGGGGSGGGGSGGGGSQAVVTQEPSLTVSPGGTVTLTCRSSTGAVTTSNYANWVQQKPGQAPRGLIGGTNKRAPGTPARFSGSLLGGKAALTLSGAQPEDEAEYYCALWYSNLWVFGGGTKLTVLEPKSSDKTHTCPPCPAPEAAGAPSVFLFPPKPKDTLMISRTPEVTCVVVDVSHEDPEVKFNWYVDGVEVHNAKTKPREEQYNSTYRVVSVLTVLHQDWLNGKEYKCKVSNKALPAPIEKTISKAKGQPREPQVYTLPPCRDELTKNQVSLWCLVKGFYPSDIAVEWESNGQPENNYKTTPPVLDSDGSFFLYSKLTVDKSRWQQGNVFSCSVMHEALHNHYTQKSLSLSPGK

SEQ ID NO: 6 - protein, 347 aa, synthetic construct
QVQLVESGGGVVQPGGSLRLSCAASGLFFASSDMSWFRQAPGKGRELVAEITSVGNNIKYADSVEGRFTISRDNSKNTVYLQMNSLRAEDTAVYYCSARRRVRYWGQGTLVTVSSEPKSSDKTHTCPPCPAPEAAGAPSVFLFPPKPKDTLMISRTPEVTCVVVDVSHEDPEVKFNWYVDGVEVHNAKTKPREEQYNSTYRVVSVLTVLHQDWLNGKEYKCKVSNKALPAPIEKTISKAKGQPREPQVCTLPPSRDELTKNQVSLSCAVKGFYPSDIAVEWESNGQPENNYKTTPPVLDSDGSFFLVSKLTVDKSRWQQGNVFSCSVMHEALHNRYTQKSLSLSPGK

SEQ ID NO: 7 - protein, 213 aa, synthetic construct
DIQLTQSPSSLSASVGDRVTITCSASSGVSHMHWYQQKPGKAPKRWIYDTSKLTSGVPSRFSGSGSGTDFTLTISSLQPEDFATYYCQQWSRNPWTFGQGTKVEIKRTVAAPSVFIFPPSDEQLKSGTASVVCLLNNFYPREAKVQWKVDNALQSGNSQESVTEQDSKDSTYSLSSTLTLSKADYEKHKVYACEVTHQGLSSPVTKSFNRGEC

SEQ ID NO: 8 - protein, 574 aa, synthetic construct
QVQLVQSGAEVKKPGASVKVSCKASGFTFRSSYISWVRQAPGQGLEWIAWIYAGSGNADYNQKFTGRVTMTVDTSTSTVYMELSSLRSEDTAVYYCARHYDPPHYFDYWGQGTLVTVSSASTKGPSVFPLAPSSKSTSGGTAALGCLVKDYFPEPVTVSWNSGALTSGVHTFPAVLQSSGLYSLSSVVTVPSSSLGTQTYICNVNHKPSNTKVDKKVEPKSCGGGGSQVQLVESGGGVVQPGGSLRLSCAASGLFFASSDMSWFRQAPGKGRELVAEITSVGNNIKYADSVEGRFTISRDNSKNTVYLQMNSLRAEDTAVYYCSARRRVRYWGQGTLVTVSSEPKSSDKTHTCPPCPAPEAAGAPSVFLFPPKPKDTLMISRTPEVTCVVVDVSHEDPEVKFNWYVDGVEVHNAKTKPREEQYNSTYRVVSVLTVLHQDWLNGKEYKCKVSNKALPAPIEKTISKAKGQPREPQVCTLPPSRDELTKNQVSLSCAVKGFYPSDIAVEWESNGQPENNYKTTPPVLDSDGSFFLVSKLTVDKSRWQQGNVFSCSVMHEALHNRYTQKSLSLSPGK

SEQ ID NO: 9 - protein, 449 aa, synthetic construct
QVQLVQSGAEVKKPGASVKVSCKASGFTFRSSYISWVRQAPGQGLEWIAWIYAGSGNADYNQKFTGRVTMTVDTSTSTVYMELSSLRSEDTAVYYCARHYDPPHYFDYWGQGTLVTVSSASTKGPSVFPLAPSSKSTSGGTAALGCLVKDYFPEPVTVSWNSGALTSGVHTFPAVLQSSGLYSLSSVVTVPSSSLGTQTYICNVNHKPSNTKVDKKVEPKSCDKTHTCPPCPAPELLGGPSVFLFPPKPKDTLMISRTPEVTCVVVDVSHEDPEVKFNWYVDGVEVHNAKTKPREEQYNSTYRVVSVLTVLHQDWLNGKEYKCKVSNKALPAPIEKTISKAKGQPREPQVYTLPPSRDELTKNQVSLTCLVKGFYPSDIAVEWESNGQPENNYKTTPPVLDSDGSFFLYSKLTVDKSRWQQGNVFSCSVMHEALHNHYTQKSLSLSPGK

SEQ ID NO: 10 - protein, 115 aa, synthetic construct
QVQLVESGGGVVQPGGSLRLSCAASGLFFASSDMSWFRQAPGKGRELVAEITSVGNNIKYADSVEGRFTISRDNSKNTVYLQMNSLRAEDTAVYYCSARRRVRYWGQGTLVTVSS

SEQ ID NO: 11 - protein, 455 aa, synthetic construct
EVKLVESGGGLVQPGGSLKLSCAASGFTFNTYAMNWVRQAPGKGLEWVARIRSKYNNYATYYADSVKDRFTISRDDAKNTLYLQMNNLRTEDTAVYYCVRHGNFGNSYVSWFAYWGQGTLVTVSSASTKGPSVFPLAPSSKSTSGGTAALGCLVKDYFPEPVTVSWNSGALTSGVHTFPAVLQSSGLYSLSSVVTVPSSSLGTQTYICNVNHKPSNTKVDKKVEPKSCDKTHTCPPCPAPEAAGGPSVFLFPPKPKDTLMISRTPEVTCVVVDVSHEDPEVKFNWYVDGVEVHNAKTKPREEQYNSTYRVVSVLTVLHQDWLNGKEYKCKVSNKALPAPIEKTISKAKGQPREPQVYTLPPSRDELTKNQVSLTCLVKGFYPSDIAVEWESNGQPENNYKTTPPVLDSDGSFFLYSKLTVDKSRWQQGNVFSCSVMHEALHNHYTQKSLSLSPGK

SEQ ID NO: 12 - protein, 214 aa, synthetic construct
QAVVTQEPSLTVSPGGTVTLTCRSSTGAVTTSNYANWVQQKPGQAPRGLIGGTNKRAPGTPARFSGSLLGGKAALTLSGAQPEDEAEYYCALWYSNLWVFGGGTKLTVLGQPKANPTVTLFPPSSEELQANKATLVCLISDFYPGAVTVAWKADSSPVKAGVETTTPSKQSNNKYAASSYLSLTPEQWKSHRSYSCQVTHEGSTVEKTVAPTEC

SEQ ID NO: 13 - protein, 249 aa, synthetic construct
EVKLVESGGGLVQPGGSLKLSCAASGFTFNTYAMNWVRQAPGKGLEWVARIRSKYNNYATYYADSVKDRFTISRDDAKNTLYLQMNNLRTEDTAVYYCVRHGNFGNSYVSWFAYWGQGTLVTVSSGGGGSGGGGSGGGGSQAVVTQEPSLTVSPGGTVTLTCRSSTGAVTTSNYANWVQQKPGQAPRGLIGGTNKRAPGTPARFSGSLLGGKAALTLSGAQPEDEAEYYCALWYSNLWVFGGGTKLTVL

SEQ ID NO: 14 - protein, 119 aa, synthetic construct
QVQLVQSGAEVKKPGASVKVSCKASGFTFRSSYISWVRQAPGQGLEWIAWIYAGSGNADYNQKFTGRVTMTVDTSTSTVYMELSSLRSEDTAVYYCARHYDPPHYFDYWGQGTLVTVSS

SEQ ID NO: 15 - protein, 106 aa, synthetic construct
DIQLTQSPSSLSASVGDRVTITCSASSGVSHMHWYQQKPGKAPKRWIYDTSKLTSGVPSRFSGSGSGTDFTLTISSLQPEDFATYYCQQWSRNPWTFGQGTKVEIK

SEQ ID NO: 16 - protein, 5 aa, synthetic construct
SSYIS

SEQ ID NO: 17 - protein, 17 aa, synthetic construct
WIYAGSGNADYNQKFTG

SEQ ID NO: 18 - protein, 10 aa, synthetic construct
HYDPPHYFDY

SEQ ID NO: 19 - protein, 10 aa, synthetic construct
SASSGVSHMH

SEQ ID NO: 20 - protein, 7 aa, synthetic construct
DTSKLTS

SEQ ID NO: 21 - protein, 9 aa, synthetic construct
QQWSRNPWT

SEQ ID NO: 22 - protein, 5 aa, synthetic construct
SSDMS

SEQ ID NO: 23 - protein, 17 aa, synthetic construct
EITSVGNNIKYADSVEG

SEQ ID NO: 24 - protein, 6 aa, synthetic construct
RRRVRY

SEQ ID NO: 25 - protein, 125 aa, synthetic construct
EVKLVESGGGLVQPGGSLKLSCAASGFTFNTYAMNWVRQAPGKGLEWVARIRSKYNNYATYYADSVKDRFTISRDDAKNTLYLQMNNLRTEDTAVYYCVRHGNFGNSYVSWFAYWGQGTLVTVSS

SEQ ID NO: 26 - protein, 109 aa, synthetic construct
QAVVTQEPSLTVSPGGTVTLTCRSSTGAVTTSNYANWVQQKPGQAPRGLIGGTNKRAPGTPARFSGSLLGGKAALTLSGAQPEDEAEYYCALWYSNLWVFGGGTKLTVL

SEQ ID NO: 27 - protein, 5 aa, synthetic construct
TYAMN

SEQ ID NO: 28 - protein, 19 aa, synthetic construct
RIRSKYNNYATYYADSVKD

SEQ ID NO: 29 - protein, 14 aa, synthetic construct
HGNFGNSYVSWFAY

SEQ ID NO: 30 - protein, 14 aa, synthetic construct
RSSTGAVTTSNYAN

SEQ ID NO: 31 - protein, 7 aa, synthetic construct
GTNKRAP

SEQ ID NO: 32 - protein, 9 aa, synthetic construct
ALWYSNLWV

SEQ ID NO: 33 - protein, 227 aa, synthetic construct
DKTHTCPPCPAPEAAGAPSVFLFPPKPKDTLMISRTPEVTCVVVDVSHEDPEVKFNWYVDGVEVHNAKTKPREEQYNSTYRVVSVLTVLHQDWLNGKEYKCKVSNKALPAPIEKTISKAKGQPREPQVYTLPPCRDELTKNQVSLWCLVKGFYPSDIAVEWESNGQPENNYKTTPPVLDSDGSFFLYSKLTVDKSRWQQGNVFSCSVMHEALHNHYTQKSLSLSPGK

SEQ ID NO: 34 - protein, 227 aa, synthetic construct
DKTHTCPPCPAPEAAGAPSVFLFPPKPKDTLMISRTPEVTCVVVDVSHEDPEVKFNWYVDGVEVHNAKTKPREEQYNSTYRVVSVLTVLHQDWLNGKEYKCKVSNKALPAPIEKTISKAKGQPREPQVCTLPPSRDELTKNQVSLSCAVKGFYPSDIAVEWESNGQPENNYKTTPPVLDSDGSFFLVSKLTVDKSRWQQGNVFSCSVMHEALHNRYTQKSLSLSPGK

SEQ ID NO: 35 - protein, 217 aa, synthetic construct
QVQLVQSGAEVKKPGASVKVSCKASGFTFRSSYISWVRQAPGQGLEWIAWIYAGSGNADYNQKFTGRVTMTVDTSTSTVYMELSSLRSEDTAVYYCARHYDPPHYFDYWGQGTLVTVSSASTKGPSVFPLAPSSKSTSGGTAALGCLVKDYFPEPVTVSWNSGALTSGVHTFPAVLQSSGLYSLSSVVTVPSSSLGTQTYICNVNHKPSNTKVDKKV

SEQ ID NO: 36 - protein, 357 aa, Homo sapiens
MATTVPDGCRNGLKSKYYRLCDKAEAWGIVLETVATAGVVTSVAFMLTLPILVCKVQDSNRRKMLPTQFLFLLGVLGIFGLTFAFIIGLDGSTGPTRFFLFGILFSICFSCLLAHAVSLTKLVRGRKPLSLLVILGLAVGFSLVQDVIAIEYIVLTMNRTNVNVFSELSAPRRNEDFVLLLTYVLFLMALTFLMSSFTFCGSFTGWKRHGAHIYLTMLLSIAIWVAWITLLMLPDFDRRWDDTILSSALAANGWVFLLAYVSPEFWLLTKQRNPMDYPVEDAFCKPQLVKKSYGVENRAYSQEEITQGFEETGDTLYAPYSTHFQLQNQPPQKEFSIPRAHAWPSPYKDYEVKKEGS

SEQ ID NO: 37 - protein, 115 aa, Vicugna pacos
QLQLVESGGGLVQPGGSLRLSCAGSGLFFASSDMSWFRQPPGKERELVAEITSVGNNIKYADSVEGRFTISRDNAKSTVYLQMNSLKPEDTAVYYCSARRRVRYWGQGTQVTVSS

SEQ ID NO: 38 - protein, 226 aa, Homo sapiens
DKTHTCPPCPAPELLGGPSVFLFPPKPKDTLMISRTPEVTCVVVDVSHEDPEVKFNWYVDGVEVHNAKTKPREEQYNSTYRVVSVLTVLHQDWLNGKEYKCKVSNKALPAPIEKTISKAKGQPREPQVYTLPPSRDELTKNQVSLTCLVKGFYPSDIAVEWESNGQPENNYKTTPPVLDSDGSFFLYSKLTVDKSRWQQGNVFSCSVMHEALHNHYTQKSLSLSPG

SEQ ID NO: 39 - protein, 119 aa, Mus musculus
QGQMQQSGAELVKPGTSVKLSCKTSGFTFRSSYISWLQQKPGQSLEWIAWIYAGSGNTDYNQKFTGKAQLTVDTSSSTAYMQFSSLTTEDSAIYYCARHYDPPHYFDYWGQGTTLTVSS

SEQ ID NO: 40 - protein, 106 aa, Mus musculus
QIVLTQSPAIMSASPGEKVTMTCSASSGVSHMHWYQQKSGTSPKRWIYDTSKLTSGVPTRFSGTGSGTSYSLSISSMEAEDAATYYCQQWSRNPWTFGGGTKLEIK

SEQ ID NO: 41 - protein, 17 aa, Mus musculus
WIYAGSGNTDYNQKFTG

SEQ ID NO: 42 - protein, 119 aa, synthetic construct
QVQLVQSGAEVKKPGASVKVSCKASGFTFRSSYISWVRQAPGQGLEWIAWIYAGSGNTDYNQKFTGRVTMTVDTSTSTVYMELSSLRSEDTAVYYCARHYDPPHYFDYWGQGTLVTVSS